European Patent Application EP 4 428 863 A2, published September 11, 2024. Title: Methods For Determining Ploidy. Applicant: Natera, Inc. The sequence listing filed with the application follows.

SEQUENCE LISTING (2 sequences)

SEQ ID NO: 1 - DNA, 20 bp, synthetic construct
  source 1..20: mol_type = other DNA
acacgacgctcttccgatct

SEQ ID NO: 2 - DNA, 21 bp, synthetic construct
  source 1..21: mol_type = other DNA
agacgtgtgctcttccgatct